European Patent Application EP 4 197 560 A1, published June 21, 2023. Title: PHARMACEUTICAL COMPOSITION COMPRISING LONG-ACTING CONJUGATE OF TRIPLE GLUCAGON/GLP-1/GIP RECEPTOR AGONIST. Applicant: HANMI PHARM. CO., LTD. The sequence listing filed with the application follows.

SEQUENCE LISTING (123 sequences)

SEQ ID NO: 1 - protein, 30 aa, Artificial Sequence
  Trigonal agonist
  MISC_FEATURE (2): Xaa is aminoisobutyric acid (Aib)
HXQGTFTSDVSSYLDGQAAKEFIAWLVKGC

SEQ ID NO: 2 - protein, 30 aa, Artificial Sequence
  Trigonal agonist
  MISC_FEATURE (2): Xaa is aminoisobutyric acid (Aib)
HXQGTFTSDVSSYLDGQAQKEFIAWLVKGC

SEQ ID NO: 3 - protein, 41 aa, Artificial Sequence
  Trigonal agonist
  MISC_FEATURE (2): Xaa is aminoisobutyric acid (Aib)
HXQGTFTSDVSSYLLGQAAKQFIAWLVKGGGPSSGAPPPSC

SEQ ID NO: 4 - protein, 30 aa, Artificial Sequence
  Trigonal agonist
  MISC_FEATURE (2): Xaa is aminoisobutyric acid (Aib)
HXQGTFTSDVSSYLLGQQQKEFIAWLVKGC

SEQ ID NO: 5 - protein, 41 aa, Artificial Sequence
  Trigonal agonist
  MISC_FEATURE (2): Xaa is aminoisobutyric acid (Aib)
HXQGTFTSDVSSYLLGQQQKEFIAWLVKGGGPSSGAPPPSC

SEQ ID NO: 6 - protein, 30 aa, Artificial Sequence
  Trigonal agonist
  MISC_FEATURE (2): Xaa is aminoisobutyric acid (Aib)
HXQGTFTSDVSSYLDGQAAKEFVAWLLKGC

SEQ ID NO: 7 - protein, 30 aa, Artificial Sequence
  Trigonal agonist
  MISC_FEATURE (2): Xaa is aminoisobutyric acid (Aib)
HXQGTFTSDVSKYLDGQAAKEFVAWLLKGC

SEQ ID NO: 8 - protein, 30 aa, Artificial Sequence
  Trigonal agonist
  MISC_FEATURE (2): Xaa is aminoisobutyric acid (Aib)
HXQGTFTSDVSKYLDGQAAQEFVAWLLKGC

SEQ ID NO: 9 - protein, 30 aa, Artificial Sequence
  Trigonal agonist
  MISC_FEATURE (2): Xaa is aminoisobutyric acid (Aib)
HXQGTFTSDVSKYLDGQAAQEFVAWLLAGC

SEQ ID NO: 10 - protein, 41 aa, Artificial Sequence
  Trigonal agonist
  MISC_FEATURE (2): Xaa is aminoisobutyric acid (Aib)
HXQGTFTSDVSKYLDGQAAQEFVAWLLAGGGPSSGAPPPSC

SEQ ID NO: 11 - protein, 41 aa, Artificial Sequence
  Trigonal agonist
  MISC_FEATURE (1): Xaa is 4-imidazoacetyl (CA)
XGEGTFTSDLSKYLDSRRQQLFVQWLKAGGPSSGAPPPSHG

SEQ ID NO: 12 - protein, 41 aa, Artificial Sequence
  Trigonal agonist
  MISC_FEATURE (1): Xaa is 4-imidazoacetyl (CA)
XGEGTFISDLSKYMDEQAVQLFVEWLMAGGPSSGAPPPSHG

SEQ ID NO: 13 - protein, 41 aa, Artificial Sequence
  Trigonal agonist
  MISC_FEATURE (1): Xaa is 4-imidazoacetyl (CA)
XGEGTFISDYSIQLDEIAVQDFVEWLLAQKPSSGAPPPSHG

SEQ ID NO: 14 - protein, 41 aa, Artificial Sequence
  Trigonal agonist
  MISC_FEATURE (1): Xaa is 4-imidazoacetyl (CA)
XGQGTFTSDYSIQLDEIAVRDFVEWLKNGGPSSGAPPPSHG

SEQ ID NO: 15 - protein, 41 aa, Artificial Sequence
  Trigonal agonist
  MISC_FEATURE (1): Xaa is 4-imidazoacetyl (CA)
XGQGTFTSDLSKQMDEEAVRLFIEWLKNGGPSSGAPPPSHG

SEQ ID NO: 16 - protein, 41 aa, Artificial Sequence
  Trigonal agonist
  MISC_FEATURE (1): Xaa is 4-imidazoacetyl (CA)
XGQGTFTSDLSKQMDSEAQQLFIEWLKNGGPSSGAPPPSHG

SEQ ID NO: 17 - protein, 41 aa, Artificial Sequence
  Trigonal agonist
  MISC_FEATURE (1): Xaa is 4-imidazoacetyl (CA)
XGQGTFTSDLSKQMDEERAREFIEWLLAQKPSSGAPPPSHG

SEQ ID NO: 18 - protein, 41 aa, Artificial Sequence
  Trigonal agonist
  MISC_FEATURE (1): Xaa is 4-imidazoacetyl (CA)
XGQGTFTSDLSKQMDSERAREFIEWLKNTGPSSGAPPPSHG

SEQ ID NO: 19 - protein, 41 aa, Artificial Sequence
  Trigonal agonist
  MISC_FEATURE (1): Xaa is 4-imidazoacetyl (CA)
XGQGTFTSDLSIQYDSEHQRDFIEWLKDTGPSSGAPPPSHG

SEQ ID NO: 20 - protein, 41 aa, Artificial Sequence
  Trigonal agonist
  MISC_FEATURE (1): Xaa is 4-imidazoacetyl (CA)
XGQGTFTSDLSIQYEEEAQQDFVEWLKDTGPSSGAPPPSHG

SEQ ID NO: 21 - protein, 39 aa, Artificial Sequence
  Trigonal agonist
  MISC_FEATURE (2): Xaa is aminoisobutyric acid (Aib)
  MISC_FEATURE (16)..(20): amino acids at positions 16 and 20 form a ring
YXQGTFTSDYSKYLDECRAKEFVQWLLDHHPSSGQPPPS

SEQ ID NO: 22 - protein, 39 aa, Artificial Sequence
  Trigonal agonist
  MISC_FEATURE (2): Xaa is aminoisobutyric acid (Aib)
  MISC_FEATURE (16)..(20): amino acids at positions 16 and 20 form a ring
YXQGTFTSDYSKCLDEKRAKEFVQWLLDHHPSSGQPPPS

SEQ ID NO: 23 - protein, 41 aa, Artificial Sequence
  Trigonal agonist
  MISC_FEATURE (2): Xaa is aminoisobutyric acid (Aib)
  MISC_FEATURE (16)..(20): amino acids at positions 16 and 20 form a ring
YXQGTFTSDYSKYLDECRAKEFVQWLLAQKGKKNDWKHNIT

SEQ ID NO: 24 - protein, 39 aa, Artificial Sequence
  Trigonal agonist
  MISC_FEATURE (2): Xaa is aminoisobutyric acid (Aib)
  MISC_FEATURE (16)..(20): amino acids at positions 16 and 20 form a ring
YXQGTFTSDYSKYLDECRAKEFVQWLKNGGPSSGAPPPS

SEQ ID NO: 25 - protein, 39 aa, Artificial Sequence
  Trigonal agonist
  MISC_FEATURE (2): Xaa is aminoisobutyric acid (Aib)
HXQGTFTSDCSKYLDERAAQDFVQWLLDGGPSSGAPPPS

SEQ ID NO: 26 - protein, 39 aa, Artificial Sequence
  Trigonal agonist
  MISC_FEATURE (2): Xaa is aminoisobutyric acid (Aib)
HXQGTFTSDCSKYLDSRAAQDFVQWLLDGGPSSGAPPPS

SEQ ID NO: 27 - protein, 40 aa, Artificial Sequence
  Trigonal agonist
  MISC_FEATURE (2): Xaa is aminoisobutyric acid (Aib)
HXQGTFTSDYSKYLDERACQDFVQWLLDQGGPSSGAPPPS

SEQ ID NO: 28 - protein, 41 aa, Artificial Sequence
  Trigonal agonist
  MISC_FEATURE (2): Xaa is aminoisobutyric acid (Aib)
HXQGTFTSDYSKYLDEKRAQEFVCWLLAQKGKKNDWKHNIT

SEQ ID NO: 29 - protein, 30 aa, Artificial Sequence
  Trigonal agonist
  MISC_FEATURE (2): Xaa is aminoisobutyric acid (Aib)
  MISC_FEATURE (16)..(20): amino acids at positions 16 and 20 form a ring
HXQGTFTSDYSKYLDEKAAKEFVQWLLNTC

SEQ ID NO: 30 - protein, 30 aa, Artificial Sequence
  Trigonal agonist
  MISC_FEATURE (2): Xaa is aminoisobutyric acid (Aib)
  MISC_FEATURE (16)..(20): amino acids at positions 16 and 20 form a ring
HXQGTFTSDYSKYLDEKAQKEFVQWLLDTC

SEQ ID NO: 31 - protein, 29 aa, Artificial Sequence
  Trigonal agonist
  MISC_FEATURE (2): Xaa is aminoisobutyric acid (Aib)
  MISC_FEATURE (16)..(20): amino acids at positions 16 and 20 form a ring
HXQGTFTSDYSKYLDEKACKEFVQWLLAQ

SEQ ID NO: 32 - protein, 39 aa, Artificial Sequence
  Trigonal agonist
  MISC_FEATURE (2): Xaa is aminoisobutyric acid (Aib)
  MISC_FEATURE (16)..(20): amino acids at positions 16 and 20 form a ring
HXQGTFTSDYSKYLDEKACKDFVQWLLDGGPSSGAPPPS

SEQ ID NO: 33 - protein, 31 aa, Artificial Sequence
  Trigonal agonist
  MISC_FEATURE (2): Xaa is aminoisobutyric acid (Aib)
  MISC_FEATURE (16)..(20): amino acids at positions 16 and 20 form a ring
HXQGTFTSDYSIAMDEIHQKDFVNWLLAQKC

SEQ ID NO: 34 - protein, 31 aa, Artificial Sequence
  Trigonal agonist
  MISC_FEATURE (2): Xaa is aminoisobutyric acid (Aib)
  MISC_FEATURE (16)..(20): amino acids at positions 16 and 20 form a ring
HXQGTFTSDYSKYLDEKRQKEFVNWLLAQKC

SEQ ID NO: 35 - protein, 31 aa, Artificial Sequence
  Trigonal agonist
  MISC_FEATURE (2): Xaa is aminoisobutyric acid (Aib)
  MISC_FEATURE (16)..(20): amino acids at positions 16 and 20 form a ring
HXQGTFTSDYSIAMDEIHQKDFVNWLLNTKC

SEQ ID NO: 36 - protein, 40 aa, Artificial Sequence
  Trigonal agonist
  MISC_FEATURE (2): Xaa is aminoisobutyric acid (Aib)
  MISC_FEATURE (16)..(20): amino acids at positions 16 and 20 form a ring
HXQGTFTSDYSKYLCEKRQKEFVQWLLNGGPSSGAPPPSG

SEQ ID NO: 37 - protein, 40 aa, Artificial Sequence
  Trigonal agonist
  MISC_FEATURE (2): Xaa is aminoisobutyric acid (Aib)
  MISC_FEATURE (16)..(20): amino acids at positions 16 and 20 form a ring
HXQGTFTSDYSKYLDECRQKEFVQWLLNGGPSSGAPPPSG

SEQ ID NO: 38 - protein, 40 aa, Artificial Sequence
  Trigonal agonist
  MISC_FEATURE (1): Xaa is 4-imidazoacetyl (CA)
  MISC_FEATURE (2): Xaa is aminoisobutyric acid (Aib)
XXQGTFTSDKSSYLDERAAQDFVQWLLDGGPSSGAPPPSS

SEQ ID NO: 39 - protein, 40 aa, Artificial Sequence
  Trigonal agonist
  MISC_FEATURE (2): Xaa is aminoisobutyric acid (Aib)
HXQGTFTSDYSKYLDGQHAQCFVAWLLAGGGPSSGAPPPS

SEQ ID NO: 40 - protein, 39 aa, Artificial Sequence
  Trigonal agonist
  MISC_FEATURE (2): Xaa is aminoisobutyric acid (Aib)
HXQGTFTSDKSKYLDERACQDFVQWLLDGGPSSGAPPPS

SEQ ID NO: 41 - protein, 39 aa, Artificial Sequence
  Trigonal agonist
  MISC_FEATURE (2): Xaa is aminoisobutyric acid (Aib)
HXQGTFTSDKSKYLDECAAQDFVQWLLDGGPSSGAPPPS

SEQ ID NO: 42 - protein, 40 aa, Artificial Sequence
  Trigonal agonist
  MISC_FEATURE (2): Xaa is aminoisobutyric acid (Aib)
  MISC_FEATURE (16)..(20): amino acids at positions 16 and 20 form a ring
YXQGTFTSDYSKYLDEKRAKEFVQWLLDHHPSSGQPPPSC

SEQ ID NO: 43 - protein, 39 aa, Artificial Sequence
  Trigonal agonist
  MISC_FEATURE (2): Xaa is aminoisobutyric acid (Aib)
  MISC_FEATURE (16)..(20): amino acids at positions 16 and 20 form a ring
YXQGTFTSDYSKYLDEKRAKEFVQWLLDHHCSSGQPPPS

SEQ ID NO: 44 - protein, 39 aa, Artificial Sequence
  Trigonal agonist
HGQGTFTSDCSKQLDGQAAQEFVAWLLAGGPSSGAPPPS

SEQ ID NO: 45 - protein, 39 aa, Artificial Sequence
  Trigonal agonist
HGQGTFTSDCSKYMDGQAAQDFVAWLLAGGPSSGAPPPS

SEQ ID NO: 46 - protein, 39 aa, Artificial Sequence
  Trigonal agonist
HGQGTFTSDCSKYLDEQHAQEFVAWLLAGGPSSGAPPPS

SEQ ID NO: 47 - protein, 39 aa, Artificial Sequence
  Trigonal agonist
HGQGTFTSDCSKYLDGQRAQEFVAWLLAGGPSSGAPPPS

SEQ ID NO: 48 - protein, 39 aa, Artificial Sequence
  Trigonal agonist
HGQGTFTSDCSKYLDGQRAQDFVNWLLAGGPSSGAPPPS

SEQ ID NO: 49 - protein, 30 aa, Artificial Sequence
  Trigonal agonist
  MISC_FEATURE (1): Xaa is 4-imidazoacetyl (CA)
  MISC_FEATURE (2): Xaa is aminoisobutyric acid (Aib)
  MISC_FEATURE (16)..(20): amino acids at positions 16 and 20 form a ring
XXQGTFTSDYSICMDEIHQKDFVNWLLNTK

SEQ ID NO: 50 - protein, 40 aa, Artificial Sequence
  Trigonal agonist
  MISC_FEATURE (2): Xaa is aminoisobutyric acid (Aib)
  MISC_FEATURE (16)..(20): amino acids at positions 16 and 20 form a ring
HXQGTFTSDYSKYLDEKRAKEFVQWLLDHHPSSGQPPPSC

SEQ ID NO: 51 - protein, 30 aa, Artificial Sequence
  Trigonal agonist
  MISC_FEATURE (2): Xaa is aminoisobutyric acid (Aib)
  MISC_FEATURE (16)..(20): amino acids at positions 16 and 20 form a ring
HXQGTFTSDYSKYLDEKRQKEFVQWLLNTC

SEQ ID NO: 52 - protein, 30 aa, Artificial Sequence
  Trigonal agonist
  MISC_FEATURE (2): Xaa is aminoisobutyric acid (Aib)
  MISC_FEATURE (16)..(20): amino acids at positions 16 and 20 form a ring
HXQGTFTSDYSKYLDEKRQKEFVQWLLDTC

SEQ ID NO: 53 - protein, 30 aa, Artificial Sequence
  Trigonal agonist
  MISC_FEATURE (2): Xaa is aminoisobutyric acid (Aib)
  MISC_FEATURE (16)..(20): amino acids at positions 16 and 20 form a ring
HXEGTFTSDYSIAMDEIHQKDFVNWLLAQC

SEQ ID NO: 54 - protein, 30 aa, Artificial Sequence
  Trigonal agonist
  MISC_FEATURE (2): Xaa is aminoisobutyric acid (Aib)
  MISC_FEATURE (16)..(20): amino acids at positions 16 and 20 form a ring
HXEGTFTSDYSIAMDEIHQKDFVDWLLAEC

SEQ ID NO: 55 - protein, 30 aa, Artificial Sequence
  Trigonal agonist
  MISC_FEATURE (2): Xaa is aminoisobutyric acid (Aib)
  MISC_FEATURE (16)..(20): amino acids at positions 16 and 20 form a ring
HXQGTFTSDYSIAMDEIHQKDFVNWLLAQC

SEQ ID NO: 56 - protein, 30 aa, Artificial Sequence
  Trigonal agonist
  MISC_FEATURE (2): Xaa is aminoisobutyric acid (Aib)
  MISC_FEATURE (16)..(20): amino acids at positions 16 and 20 form a ring
HXQGTFTSDYSKYLDEKRQKEFVNWLLAQC

SEQ ID NO: 57 - protein, 30 aa, Artificial Sequence
  Trigonal agonist
  MISC_FEATURE (2): Xaa is aminoisobutyric acid (Aib)
  MISC_FEATURE (16)..(20): amino acids at positions 16 and 20 form a ring
HXQGTFTSDYSIAMDEIHQKDFVNWLLNTC

SEQ ID NO: 58 - protein, 31 aa, Artificial Sequence
  Trigonal agonist
  MISC_FEATURE (2): Xaa is aminoisobutyric acid (Aib)
  MISC_FEATURE (16)..(20): amino acids at positions 16 and 20 form a ring
HXQGTFTSDYSKYLDEKRQKEFVQWLLNTKC

SEQ ID NO: 59 - protein, 30 aa, Artificial Sequence
  Trigonal agonist
  MISC_FEATURE (1): Xaa is 4-imidazoacetyl (CA)
  MISC_FEATURE (2): Xaa is aminoisobutyric acid (Aib)
  MISC_FEATURE (16)..(20): amino acids at positions 16 and 20 form a ring
XXQGTFTSDYSICMDEKHQKDFVNWLLNTK

SEQ ID NO: 60 - protein, 30 aa, Artificial Sequence
  Trigonal agonist
  MISC_FEATURE (1): Xaa is 4-imidazoacetyl (CA)
  MISC_FEATURE (2): Xaa is aminoisobutyric acid (Aib)
  MISC_FEATURE (16)..(20): amino acids at positions 16 and 20 form a ring
XXQGTFTSDYSIAMDEKHCKDFVNWLLNTK

SEQ ID NO: 61 - protein, 30 aa, Artificial Sequence
  Trigonal agonist
  MISC_FEATURE (1): Xaa is 4-imidazoacetyl (CA)
  MISC_FEATURE (2): Xaa is aminoisobutyric acid (Aib)
  MISC_FEATURE (16)..(20): amino acids at positions 16 and 20 form a ring
XXQGTFTSDYSIAMDEIACKDFVNWLLNTK

SEQ ID NO: 62 - protein, 39 aa, Artificial Sequence
  Trigonal agonist
  MISC_FEATURE (1): Xaa is 4-imidazoacetyl (CA)
  MISC_FEATURE (2): Xaa is aminoisobutyric acid (Aib)
XXQGTFTSDKSKYLDERAAQDFVQWLLDGGPSSGAPPPS

SEQ ID NO: 63 - protein, 39 aa, Artificial Sequence
  Trigonal agonist
  MISC_FEATURE (1): Xaa is 4-imidazoacetyl (CA)
  MISC_FEATURE (2): Xaa is aminoisobutyric acid (Aib)
XXQGTFTSDCSKYLDERAAQDFVQWLLDGGPSSGAPPPS

SEQ ID NO: 64 - protein, 39 aa, Artificial Sequence
  Trigonal agonist
  MISC_FEATURE (2): Xaa is aminoisobutyric acid (Aib)
  MISC_FEATURE (16)..(20): amino acids at positions 16 and 20 form a ring
YXQGTFTSDYSKYLDECAAKEFVQWLLDHHPSSGQPPPS

SEQ ID NO: 65 - protein, 39 aa, Artificial Sequence
  Trigonal agonist
  MISC_FEATURE (2): Xaa is aminoisobutyric acid (Aib)
  MISC_FEATURE (16)..(20): amino acids at positions 16 and 20 form a ring
HXQGTFTSDYSKCLDEKRAKEFVQWLLDHHPSSGQPPPS

SEQ ID NO: 66 - protein, 39 aa, Artificial Sequence
  Trigonal agonist
  MISC_FEATURE (2): Xaa is aminoisobutyric acid (Aib)
  MISC_FEATURE (16)..(20): amino acids at positions 16 and 20 form a ring
YXQGTFTSDYSKYLDECRAKDFVQWLLDHHPSSGQPPPS

SEQ ID NO: 67 - protein, 39 aa, Artificial Sequence
  Trigonal agonist
  MISC_FEATURE (2): Xaa is aminoisobutyric acid (Aib)
  MISC_FEATURE (16)..(20): amino acids at positions 16 and 20 form a ring
YXQGTFTSDYSKYLDECAAKDFVQWLLDHHPSSGQPPPS

SEQ ID NO: 68 - protein, 39 aa, Artificial Sequence
  Trigonal agonist
  MISC_FEATURE (2): Xaa is aminoisobutyric acid (Aib)
  MISC_FEATURE (16)..(20): amino acids at positions 16 and 20 form a ring
YXQGTFTSDYSKCLDEKAAKEFVQWLLDHHPSSGQPPPS

SEQ ID NO: 69 - protein, 39 aa, Artificial Sequence
  Trigonal agonist
  MISC_FEATURE (2): Xaa is aminoisobutyric acid (Aib)
  MISC_FEATURE (16)..(20): amino acids at positions 16 and 20 form a ring
YXQGTFTSDYSKCLDERAAKEFVQWLLDHHPSSGQPPPS

SEQ ID NO: 70 - protein, 39 aa, Artificial Sequence
  Trigonal agonist
  MISC_FEATURE (2): Xaa is aminoisobutyric acid (Aib)
  MISC_FEATURE (16)..(20): amino acids at positions 16 and 20 form a ring
YXQGTFTSDYSKCLDEKRAKDFVQWLLDHHPSSGQPPPS

SEQ ID NO: 71 - protein, 39 aa, Artificial Sequence
  Trigonal agonist
  MISC_FEATURE (2): Xaa is aminoisobutyric acid (Aib)
  MISC_FEATURE (16)..(20): amino acids at positions 16 and 20 form a ring
YXQGTFTSDYSKYLDERACKDFVQWLLDHHPSSGQPPPS

SEQ ID NO: 72 - protein, 39 aa, Artificial Sequence
  Trigonal agonist
  MISC_FEATURE (2): Xaa is aminoisobutyric acid (Aib)
  MISC_FEATURE (16)..(20): amino acids at positions 16 and 20 form a ring
YXQGTFTSDCSKYLDERAAKDFVQWLLDHHPSSGQPPPS

SEQ ID NO: 73 - protein, 39 aa, Artificial Sequence
  Trigonal agonist
  MISC_FEATURE (1): Xaa is 4-imidazoacetyl (CA)
  MISC_FEATURE (2): Xaa is aminoisobutyric acid (Aib)
  MISC_FEATURE (16)..(20): amino acids at positions 16 and 20 form a ring
XXQGTFTSDYSKYLDECRAKEFVQWLLDHHPSSGQPPPS

SEQ ID NO: 74 - protein, 39 aa, Artificial Sequence
  Trigonal agonist
  MISC_FEATURE (1): Xaa is 4-imidazoacetyl (CA)
  MISC_FEATURE (2): Xaa is aminoisobutyric acid (Aib)
  MISC_FEATURE (16)..(20): amino acids at positions 16 and 20 form a ring
XXQGTFTSDYSKCLDEKRAKEFVQWLLDHHPSSGQPPPS

SEQ ID NO: 75 - protein, 40 aa, Artificial Sequence
  Trigonal agonist
  MISC_FEATURE (2): Xaa is aminoisobutyric acid (Aib)
  MISC_FEATURE (16)..(20): amino acids at positions 16 and 20 form a ring
YXQGTFTSDYSKYLDEKAAKEFVQWLLDHHPSSGQPPPSC

SEQ ID NO: 76 - protein, 40 aa, Artificial Sequence
  Trigonal agonist
  MISC_FEATURE (2): Xaa is aminoisobutyric acid (Aib)
  MISC_FEATURE (16)..(20): amino acids at positions 16 and 20 form a ring
YXQGTFTSDYSKYLDEKRAKDFVQWLLDHHPSSGQPPPSC

SEQ ID NO: 77 - protein, 40 aa, Artificial Sequence
  Trigonal agonist
  MISC_FEATURE (2): Xaa is aminoisobutyric acid (Aib)
  MISC_FEATURE (16)..(20): amino acids at positions 16 and 20 form a ring
YXQGTFTSDYSKYLDEKAAKDFVQWLLDHHPSSGQPPPSC

SEQ ID NO: 78 - protein, 31 aa, Artificial Sequence
  Trigonal agonist
  MISC_FEATURE (2): Xaa is aminoisobutyric acid (Aib)
  MISC_FEATURE (16)..(20): amino acids at positions 16 and 20 form a ring
HXQGTFTSDYSKYLDEKRQKEFVQWLLDTKC

SEQ ID NO: 79 - protein, 31 aa, Artificial Sequence
  Trigonal agonist
  MISC_FEATURE (2): Xaa is aminoisobutyric acid (Aib)
  MISC_FEATURE (16)..(20): amino acids at positions 16 and 20 form a ring
HXEGTFTSDYSIAMDEIHQKDFVNWLLAQKC

SEQ ID NO: 80 - protein, 31 aa, Artificial Sequence
  Trigonal agonist
  MISC_FEATURE (2): Xaa is aminoisobutyric acid (Aib)
  MISC_FEATURE (16)..(20): amino acids at positions 16 and 20 form a ring
HXEGTFTSDYSIAMDEIHQKDFVDWLLAEKC

SEQ ID NO: 81 - protein, 30 aa, Artificial Sequence
  Trigonal agonist
  MISC_FEATURE (1): Xaa is 4-imidazoacetyl (CA)
  MISC_FEATURE (2): Xaa is aminoisobutyric acid (Aib)
  MISC_FEATURE (16)..(20): amino acids at positions 16 and 20 form a ring
XXQGTFTSDYSKYLDEKRQKEFVQWLLNTC

SEQ ID NO: 82 - protein, 30 aa, Artificial Sequence
  Trigonal agonist
  MISC_FEATURE (1): Xaa is 4-imidazoacetyl (CA)
  MISC_FEATURE (2): Xaa is aminoisobutyric acid (Aib)
  MISC_FEATURE (16)..(20): amino acids at positions 16 and 20 form a ring
XXQGTFTSDYSKYLDEKRQKEFVQWLLDTC

SEQ ID NO: 83 - protein, 30 aa, Artificial Sequence
  Trigonal agonist
  MISC_FEATURE (1): Xaa is 4-imidazoacetyl (CA)
  MISC_FEATURE (2): Xaa is aminoisobutyric acid (Aib)
  MISC_FEATURE (16)..(20): amino acids at positions 16 and 20 form a ring
XXEGTFTSDYSIAMDEIHQKDFVNWLLAQC

SEQ ID NO: 84 - protein, 30 aa, Artificial Sequence
  Trigonal agonist
  MISC_FEATURE (1): Xaa is 4-imidazoacetyl (CA)
  MISC_FEATURE (2): Xaa is aminoisobutyric acid (Aib)
  MISC_FEATURE (16)..(20): amino acids at positions 16 and 20 form a ring
XXEGTFTSDYSIAMDEIHQKDFVDWLLAEC

SEQ ID NO: 85 - protein, 30 aa, Artificial Sequence
  Trigonal agonist
  MISC_FEATURE (1): Xaa is 4-imidazoacetyl (CA)
  MISC_FEATURE (2): Xaa is aminoisobutyric acid (Aib)
  MISC_FEATURE (16)..(20): amino acids at positions 16 and 20 form a ring
XXQGTFTSDYSIAMDEIHQKDFVNWLLAQC

SEQ ID NO: 86 - protein, 30 aa, Artificial Sequence
  Trigonal agonist
  MISC_FEATURE (1): Xaa is 4-imidazoacetyl (CA)
  MISC_FEATURE (2): Xaa is aminoisobutyric acid (Aib)
  MISC_FEATURE (16)..(20): amino acids at positions 16 and 20 form a ring
XXQGTFTSDYSKYLDEKRQKEFVNWLLAQC

SEQ ID NO: 87 - protein, 30 aa, Artificial Sequence
  Trigonal agonist
  MISC_FEATURE (1): Xaa is 4-imidazoacetyl (CA)
  MISC_FEATURE (2): Xaa is aminoisobutyric acid (Aib)
  MISC_FEATURE (16)..(20): amino acids at positions 16 and 20 form a ring
XXQGTFTSDYSIAMDEIHQKDFVNWLLNTC

SEQ ID NO: 88 - protein, 31 aa, Artificial Sequence
  Trigonal agonist
  MISC_FEATURE (1): Xaa is 4-imidazoacetyl (CA)
  MISC_FEATURE (2): Xaa is aminoisobutyric acid (Aib)
  MISC_FEATURE (16)..(20): amino acids at positions 16 and 20 form a ring
XXQGTFTSDYSKYLDEKRQKEFVQWLLNTKC

SEQ ID NO: 89 - protein, 31 aa, Artificial Sequence
  Trigonal agonist
  MISC_FEATURE (1): Xaa is 4-imidazoacetyl (CA)
  MISC_FEATURE (2): Xaa is aminoisobutyric acid (Aib)
  MISC_FEATURE (16)..(20): amino acids at positions 16 and 20 form a ring
XXQGTFTSDYSKYLDEKRQKEFVQWLLDTKC

SEQ ID NO: 90 - protein, 31 aa, Artificial Sequence
  Trigonal agonist
  MISC_FEATURE (1): Xaa is 4-imidazoacetyl (CA)
  MISC_FEATURE (2): Xaa is aminoisobutyric acid (Aib)
  MISC_FEATURE (16)..(20): amino acids at positions 16 and 20 form a ring
XXEGTFTSDYSIAMDEIHQKDFVNWLLAQKC

SEQ ID NO: 91 - protein, 31 aa, Artificial Sequence
  Trigonal agonist
  MISC_FEATURE (1): Xaa is 4-imidazoacetyl (CA)
  MISC_FEATURE (2): Xaa is aminoisobutyric acid (Aib)
  MISC_FEATURE (16)..(20): amino acids at positions 16 and 20 form a ring
XXEGTFTSDYSIAMDEIHQKDFVDWLLAEKC

SEQ ID NO: 92 - protein, 31 aa, Artificial Sequence
  Trigonal agonist
  MISC_FEATURE (1): Xaa is 4-imidazoacetyl (CA)
  MISC_FEATURE (2): Xaa is aminoisobutyric acid (Aib)
  MISC_FEATURE (16)..(20): amino acids at positions 16 and 20 form a ring
XXQGTFTSDYSIAMDEIHQKDFVNWLLAQKC

SEQ ID NO: 93 - protein, 31 aa, Artificial Sequence
  Trigonal agonist
  MISC_FEATURE (1): Xaa is 4-imidazoacetyl (CA)
  MISC_FEATURE (2): Xaa is aminoisobutyric acid (Aib)
  MISC_FEATURE (16)..(20): amino acids at positions 16 and 20 form a ring
XXQGTFTSDYSKYLDEKRQKEFVNWLLAQKC

SEQ ID NO: 94 - protein, 31 aa, Artificial Sequence
  Trigonal agonist
  MISC_FEATURE (1): Xaa is 4-imidazoacetyl (CA)
  MISC_FEATURE (2): Xaa is aminoisobutyric acid (Aib)
  MISC_FEATURE (16)..(20): amino acids at positions 16 and 20 form a ring
XXQGTFTSDYSIAMDEIHQKDFVNWLLNTKC

SEQ ID NO: 95 - protein, 39 aa, Artificial Sequence
  Trigonal agonist
  MISC_FEATURE (2): Xaa is aminoisobutyric acid (Aib)
  MISC_FEATURE (16)..(20): amino acids at positions 16 and 20 form a ring
YXQGTFTSDYSKYLDEKRAKEFVQWLLCHHPSSGQPPPS

SEQ ID NO: 96 - protein, 39 aa, Artificial Sequence
  Trigonal agonist
  MISC_FEATURE (2): Xaa is aminoisobutyric acid (Aib)
  MISC_FEATURE (16)..(20): amino acids at positions 16 and 20 form a ring
YXQGTFTSDYSKYLDEKRAKEFVQWLLDHCPSSGQPPPS

SEQ ID NO: 97 - protein, 39 aa, Artificial Sequence
  Trigonal agonist
  MISC_FEATURE (2): Xaa is aminoisobutyric acid (Aib)
  MISC_FEATURE (16)..(20): amino acids at positions 16 and 20 form a ring
YXQGTFTSDYSKYLDEKRAKEFVQWLLDCHPSSGQPPPS

SEQ ID NO: 98 - protein, 40 aa, Artificial Sequence
  Trigonal agonist
  MISC_FEATURE (2): Xaa is aminoisobutyric acid (Aib)
  MISC_FEATURE (16)..(20): amino acids at positions 16 and 20 form a ring
YXQGTFTSDYSKALDEKAAKEFVNWLLDHHPSSGQPPPSC

SEQ ID NO: 99 - protein, 40 aa, Artificial Sequence
  Trigonal agonist
  MISC_FEATURE (2): Xaa is aminoisobutyric acid (Aib)
  MISC_FEATURE (16)..(20): amino acids at positions 16 and 20 form a ring
YXQGTFTSDYSKALDEKAAKDFVNWLLDHHPSSGQPPPSC

SEQ ID NO: 100 - protein, 40 aa, Artificial Sequence
  Trigonal agonist
  MISC_FEATURE (2): Xaa is aminoisobutyric acid (Aib)
  MISC_FEATURE (16)..(20): amino acids at positions 16 and 20 form a ring
YXQGTFTSDYSKALDEKAAKEFVQWLLDQHPSSGQPPPSC

SEQ ID NO: 101 - protein, 40 aa, Artificial Sequence
  Trigonal agonist
  MISC_FEATURE (2): Xaa is aminoisobutyric acid (Aib)
  MISC_FEATURE (16)..(20): amino acids at positions 16 and 20 form a ring
YXQGTFTSDYSKALDEKAAKEFVNWLLDQHPSSGQPPPSC

SEQ ID NO: 102 - protein, 40 aa, Artificial Sequence
  Trigonal agonist
  MISC_FEATURE (2): Xaa is aminoisobutyric acid (Aib)
  MISC_FEATURE (16)..(20): amino acids at positions 16 and 20 form a ring
YXQGTFTSDYSKALDEKAAKDFVNWLLDQHPSSGQPPPSC

SEQ ID NO: 103 - protein, 12 aa, HOMO SAPIENS
ESKYGPPCPSCP

SEQ ID NO: 104 - protein, 11 aa, Artificial Sequence
  Variant of hinge region
ESKYGPPPSCP

SEQ ID NO: 105 - protein, 11 aa, Artificial Sequence
  Variant of hinge region
ESKYGPPCPSP

SEQ ID NO: 106 - protein, 10 aa, Artificial Sequence
  Variant of hinge region
ESKYGPPCPS

SEQ ID NO: 107 - protein, 10 aa, Artificial Sequence
  Variant of hinge region
ESKYGPPCPP

SEQ ID NO: 108 - protein, 8 aa, Artificial Sequence
  Variant of hinge region
KYGPPCPS

SEQ ID NO: 109 - protein, 8 aa, Artificial Sequence
  Variant of hinge region
ESKYGPPC

SEQ ID NO: 110 - protein, 7 aa, Artificial Sequence
  Variant of hinge region
EKYGPPC

SEQ ID NO: 111 - protein, 6 aa, Artificial Sequence
  Variant of hinge region
ESPSCP

SEQ ID NO: 112 - protein, 5 aa, Artificial Sequence
  Variant of hinge region
EPSCP

SEQ ID NO: 113 - protein, 4 aa, Artificial Sequence
  Variant of hinge region
PSCP

SEQ ID NO: 114 - protein, 10 aa, Artificial Sequence
  Variant of hinge region
ESKYGPPSCP

SEQ ID NO: 115 - protein, 9 aa, Artificial Sequence
  Variant of hinge region
KYGPPPSCP

SEQ ID NO: 116 - protein, 9 aa, Artificial Sequence
  Variant of hinge region
ESKYGPSCP

SEQ ID NO: 117 - protein, 8 aa, Artificial Sequence
  Variant of hinge region
ESKYGPPC

SEQ ID NO: 118 - protein, 7 aa, Artificial Sequence
  Variant of hinge region
KYGPPCP

SEQ ID NO: 119 - protein, 7 aa, Artificial Sequence
  Variant of hinge region
ESKPSCP

SEQ ID NO: 120 - protein, 6 aa, Artificial Sequence
  Variant of hinge region
ESPSCP

SEQ ID NO: 121 - protein, 4 aa, Artificial Sequence
  Variant of hinge region
EPSC

SEQ ID NO: 122 - protein, 3 aa, Artificial Sequence
  Variant of hinge region
SCP

SEQ ID NO: 123 - protein, 221 aa, homo sapiens
PSCPAPEFLGGPSVFLFPPKPKDTLMISRTPEVTCVVVDVSQEDPEVQFNWYVDGVEVHNAKTKPREEQFNSTYRVVSVLTVLHQDWLNGKEYKCKVSNKGLPSSIEKTISKAKGQPREPQVYTLPPSQEEMTKNQVSLTCLVKGFYPSDIAVEWESNGQPENNYKTTPPVLDSDGSFFLYSRLTVDKSRWQEGNVFSCSVMHEALHNHYTQKSLSLSLGK